European Patent Application EP 4 792 825 A1, published August 19, 2026. Title: Il‑4 and SDF‑1 derived peptides for enhancing skeletal muscle repair. Applicant: University of Warsaw. Application PL -, filed January 16, 2025. The sequence listing filed with the application follows.

SEQUENCE LISTING (16 sequences)

SEQ ID NO: 1 - protein, 12 aa, synthetic construct
  MOD_RES >12: note = AMIDATION
LITLQEIIKTLN

SEQ ID NO: 2 - protein, 16 aa, synthetic construct
  MOD_RES >16: note = AMIDATION
LQLIRFLKRLDRNLWG

SEQ ID NO: 3 - protein, 9 aa, synthetic construct
  MOD_RES >9: note = AMIDATION
LKPVSLSYR

SEQ ID NO: 4 - protein, 12 aa, synthetic construct
  MOD_RES >12: note = AMIDATION
LVARLKNNNRQV

SEQ ID NO: 5 - protein, 4 aa, synthetic construct
  MOD_RES >4: note = AMIDATION
LRGD

SEQ ID NO: 6 - skipped

SEQ ID NO: 7 - protein, 4 aa, synthetic construct
VLGL

SEQ ID NO: 8 - protein, 4 aa, synthetic construct
PLGL

SEQ ID NO: 9 - protein, 4 aa, synthetic construct
PAGL

SEQ ID NO: 10 - protein, 4 aa, synthetic construct
PLNL

SEQ ID NO: 11 - protein, 4 aa, synthetic construct
PANL

SEQ ID NO: 12 - protein, 4 aa, synthetic construct
VALL

SEQ ID NO: 13 - protein, 11 aa, synthetic construct
ITLQEIIKTLN

SEQ ID NO: 14 - protein, 15 aa, synthetic construct
QLIRFLKRLDRNLWG

SEQ ID NO: 15 - protein, 8 aa, synthetic construct
KPVSLSYR

SEQ ID NO: 16 - protein, 11 aa, synthetic construct
VARLKNNNRQV